European Patent Application EP 4 606 822 A1, published August 27, 2025. Title: 抗体-药物偶联物及其制备方法和在抗肿瘤中的用途. Applicant: 普众发现医药科技（上海）有限公司. Application CN. The sequence listing filed with the application follows.

SEQUENCE LISTING (18 sequences)

SEQ ID NO: 1 - protein, 11 aa, synthetic construct
RASQSISDYLH

SEQ ID NO: 2 - protein, 7 aa, synthetic construct
YASQSIS

SEQ ID NO: 3 - protein, 9 aa, synthetic construct
QSGRSFPLT

SEQ ID NO: 4 - protein, 7 aa, synthetic construct
TGNYRWS

SEQ ID NO: 5 - protein, 16 aa, synthetic construct
CIYYSGAITYTPSLTG

SEQ ID NO: 6 - protein, 13 aa, synthetic construct
DGGTVVEGWYFDV

SEQ ID NO: 7 - protein, 16 aa, synthetic construct
NIYYSGAITYNPSLKS

SEQ ID NO: 8 - protein, 16 aa, synthetic construct
YIYYSGAITYNPSLKS

SEQ ID NO: 9 - protein, 107 aa, synthetic construct
DIVMTQSPATLSVTPGDRVSLSCRASQSISDYLHWYQQKSHESPRLLIKYASQSISGIPSRFSGSGSGSDFTLNINSVEPEDVGLYYCQSGRSFPLTFGAGTKVELK

SEQ ID NO: 10 - protein, 123 aa, synthetic construct
DVQLQESGPGLVKPSQTVSLTCTVTGISITTGNYRWSWIRQFPGNKLEWIGCIYYSGAITYTPSLTGRTTITRDTSRNQFFLEMNSLTAEDTATYYCARDGGTVVEGWYFDVWGAGTTVTVSS

SEQ ID NO: 11 - protein, 107 aa, synthetic construct
EIVLTQSPDTQSVTPKEKVTITCRASQSISDYLHWYQQKPDQSPKLLIKYASQSISGVPSRFSGSGSGTDFTLTINSLEAEDAATYYCQSGRSFPLTFGGGTKVEIK

SEQ ID NO: 12 - protein, 107 aa, synthetic construct
EIVLTQSPDTQSVTPKEKVTITCRASQSISDYLHWYQQKPDQSPKLLIKYASQSISGVPSRFSGSGSGTDFTLTINSLEAEDVGLYYCQSGRSFPLTFGGGTKVEIK

SEQ ID NO: 13 - protein, 107 aa, synthetic construct
EIVLTQSPDTQSVTPKEKVTITCRASQSISDYLHWYQQKPGQAPKLLIKYASQSISGVPSRFSGSGSGTDFTLTINSLEAEDFGLYYCQSGRSFPLTFGGGTKVEIK

SEQ ID NO: 14 - protein, 123 aa, synthetic construct
QVQLQESGPGLVKPSQTLSLTCTVSGISITTGNYRWSWIRQHPGKKLEWIGNIYYSGAITYNPSLKSRVTISRDTSKNQFFLKLSSVTAADTAVYYCARDGGTVVEGWYFDVWGKGTTVTVSS

SEQ ID NO: 15 - protein, 123 aa, synthetic construct
QVQLQESGPGLVKPSQTVSLTCTVSGISITTGNYRWSWIRQHPGKKLEWIGNIYYSGAITYNPSLKSRVTISRDTSKNQFFLKLSSVTAADTAVYYCARDGGTVVEGWYFDVWGKGTTVTVSS

SEQ ID NO: 16 - protein, 123 aa, synthetic construct
QVQLQESGPGLVKPSQTLSLTCTVSGISITTGNYRWSWIRQPPGKGLEWIGYIYYSGAITYNPSLKSRVTISRDTSKNQFSLQLRSVTAADTAVYYCARDGGTVVEGWYFDVWGQGTTVTVSS

SEQ ID NO: 17 - protein, 330 aa, synthetic construct [sequence omitted]

SEQ ID NO: 18 - protein, 107 aa, synthetic construct [sequence omitted]